European Patent Specification EP 3 541 840 B1, published December 27, 2023. Title: Anti-HLA-G antibodies and use thereof. Applicant: F. Hoffmann-La Roche AG. The sequence listing filed with the application follows.

SEQUENCE LISTING (39 sequences)

SEQ ID NO: 1 - protein, 5 aa, rat
SYDMH

SEQ ID NO: 2 - protein, 17 aa, rat
WIYPGNGNTKYNQKFNG

SEQ ID NO: 3 - protein, 12 aa, rat
PTVATRYNWFAY

SEQ ID NO: 4 - protein, 10 aa, rat
SASSSVNYMH

SEQ ID NO: 5 - protein, 7 aa, rat
LTSNLAS

SEQ ID NO: 6 - protein, 10 aa, rat
QQWSSNLPIT

SEQ ID NO: 7 - protein, 121 aa, rat
QVQLQQSGAELVKPGSSVKISCKASGYSFPSYDMHWIKQQPGNGLEWIGWIYPGNGNTKYNQKFNGKASLTADKSSSTAYMQLSSLTSEDSAVYFCAKPTVATRYNWFAYWGQGTLVTVSS

SEQ ID NO: 8 - protein, 107 aa, rat
QIVLTQSPALMSASPGEKVTMTCSASSSVNYMHWYQQKPRSSPKPWIYLTSNLASGVPARFSGSGSGTSYSLTISTMEAEDAATYYCQQWSSNLPITFGSGTKLEIK

SEQ ID NO: 9 - protein, 5 aa, rat
TYSVS

SEQ ID NO: 10 - protein, 16 aa, rat
AIWSGGSTDYNSALKS

SEQ ID NO: 11 - protein, 12 aa, rat
MNNKFGYWYFDL

SEQ ID NO: 12 - protein, 11 aa, rat
RASETVSTMLH

SEQ ID NO: 13 - protein, 7 aa, rat
LASHLES

SEQ ID NO: 14 - protein, 9 aa, rat
QQTWNDPLT

SEQ ID NO: 15 - protein, 120 aa, rat
QVQLKESGPGLVQPSQTLSLTCSVSGFSLTTYSVSWVRQPPGKGLEWIGAIWSGGSTDYNSALKSRLRISRDTSKSQVLLKMNSLQTEDRAMYFCVRMNNKFGYWYFDLWGPGTMVTVSS

SEQ ID NO: 16 - protein, 106 aa, rat
DTVLTQSPTLAVSPGEKITISCRASETVSTMLHWYQQKPGQQPKLLISLASHLESGVPARFTGSGSGTDFTLTIDPVEADDTATYYCQQTWNDPLTFGSGTKLEIK

SEQ ID NO: 17 - protein, 314 aa, homo sapiens
GSHSMRYFSAAVSRPGRGEPRFIAMGYVDDTQFVRFDSDSACPRMEPRAPWVEQEGPEYWEEETRNTKAHAQTDRMNLQTLRGYYNQSEASSHTLQWMIGCDLGSDGRLLRGYEQYAYDGKDYLALNEDLRSWTAADTAAQISKRKCEAANVAEQRRAYLEGTCVEWLHRYLENGKEMLQRADPPKTHVTHHPVFDYEATLRCWALGFYPAEIILTWQRDGEDQTQDVELVETRPAGDGTFQKWAAVVVPSGEEQRYTCHVQHEGLPEPLMLRWKQSSLPTIPIMGIVAGLVVLAAVVTGAAVAAVLWRKKSSD

SEQ ID NO: 18 - protein, 274 aa, homo sapiens
GSHSMRYFSAAVSRPGRGEPRFIAMGYVDDTQFVRFDSDSACPRMEPRAPWVEQEGPEYWEEETRNTKAHAQTDRMNLQTLRGYYNQSEASSHTLQWMIGCDLGSDGRLLRGYEQYAYDGKDYLALNEDLRSWTAADTAAQISKRKCEAANVAEQRRAYLEGTCVEWLHRYLENGKEMLQRADPPKTHVTHHPVFDYEATLRCWALGFYPAEIILTWQRDGEDQTQDVELVETRPAGDGTFQKWAAVVVPSGEEQRYTCHVQHEGLPEPLMLRW

SEQ ID NO: 19 - protein, 99 aa, homo sapiens [sequence omitted]

SEQ ID NO: 20 - protein, 275 aa, Artificial
  modified human HLA-G (wherein the HLA-G specific amino acids have been replaced by HLA-A consensus amino acids  (= degrafted HLA-G) ECD
GSHSMRYFSAAVSRPGRGEPRFIAMGYVDDTQFVRFDSDAASPRMEPRAPWVEQEGPEYWDEETRNTKAHAQTDRVNLGTLRGCYNQSEAGSHTLQWMIGCDVGSDGRLLRGYEQYAYDGKDYLALNEDLRSWTAADTAAQISKRKCEAAHVAEQRRAYLEGTCVEWLRRYLENGKETLQRADPPKTHVTHHPVSDHEATLRCWALGFYPAEITLTWQRDGEDQTQDVELVETRPAGDGTFQKWAAVVVPSGEEQRYTCHVQHEGLPEPLTLRWK

SEQ ID NO: 21 - protein, 341 aa, homo sapiens
GSHSMRYFFTSVSRPGRGEPRFIAVGYVDDTQFVRFDSDAASQRMEPRAPWIEQEGPEYWDGETRKVKAHSQTHRVDLGTLRGYYNQSEAGSHTVQRMYGCDVGSDWRFLRGYHQYAYDGKDYIALKEDLRSWTAADMAAQTTKHKWEAAHVAEQLRAYLEGTCVEWLRRYLENGKETLQRTDAPKTHMTHHAVSDHEATLRCWALSFYPAEITLTWQRDGEDQTQDTELVETRPAGDGTFQKWAAVVVPSGQEQRYTCHVQHEGLPKPLTLRWEPSSQPTIPIVGIIAGLVLFGAVITGAVVAAVMWRRKSSDRKGGSYSQAASSDSAQGSDVSLTACKV

SEQ ID NO: 22 - protein, 275 aa, homo sapiens [sequence omitted]

SEQ ID NO: 23 - protein, 275 aa, mus musculus
GPHSLRYFVTAVSRPGLGEPRFIAVGYVDDTQFVRFDSDADNPRFEPRAPWMEQEGPEYWEEQTQRAKSDEQWFRVSLRTAQRCYNQSKGGSHTFQRMFGCDVGSDWRLLRGYQQFAYDGRDYIALNEDLKTWTAADTAALITRRKWEQAGDAEYYRAYLEGECVEWLRRYLELGNETLLRTDSPKAHVTYHPRSQVDVTLRCWALGFYPADITLTWQLNGEDLTQDMELVETRPAGDGTFQKWAAVVVPLGKEQNYTCHVHHKGLPEPLTLRWK

SEQ ID NO: 24 - protein, 274 aa, rat
GSHSLRYFYTAVSRPGLGEPRFIAVGYVDDTEFVRFDSDAENPRMEPRARWMEREGPEYWEQQTRIAKEWEQIYRVDLRTLRGCYNQSEGGSHTIQEMYGCDVGSDGSLLRGYRQDAYDGRDYIALNEDLKTWTAADFAAQITRNKWERARYAERLRAYLEGTCVEWLSRYLELGKETLLRSDPPEAHVTLHPRPEGDVTLRCWALGFYPADITLTWQLNGEDLTQDMELVETRPAGDGTFQKWASVVVPLGKEQNYTCRVEHEGLPKPLSQRW

SEQ ID NO: 25 - protein, 440 aa, homo sapiens
RIIPRHLQLGCGGSGGGGSGGGGSIQRTPKIQVYSRHPAENGKSNFLNCYVSGFHPSDIEVDLLKNGERIEKVEHSDLSFSKDWSFYLLYYTEFTPTEKDEYACRVNHVTLSQPKIVKWDRDMGGGGSGGGGSGGGGSGGGGSGSHSMRYFSAAVSRPGRGEPRFIAMGYVDDTQFVRFDSDSACPRMEPRAPWVEQEGPEYWEEETRNTKAHAQTDRMNLQTLRGCYNQSEASSHTLQWMIGCDLGSDGRLLRGYEQYAYDGKDYLALNEDLRSWTAADTAAQISKRKCEAANVAEQRRAYLEGTCVEWLHRYLENGKEMLQRADPPKTHVTHHPVFDYEATLRCWALGFYPAEIILTWQRDGEDQTQDVELVETRPAGDGTFQKWAAVVVPSGEEQRYTCHVQHEGLPEPLMLRWGSGLNDIFEAQKIEWHEHHHHHH

SEQ ID NO: 26 - protein, 441 aa, Artificial
  exemplary modified human HLA-G ß2M MHC class I complex (wherein the HLA-G specific amino acids have been replaced by HLA-A consensus amino acids  (= degrafted HLA-G)
RIIPRHLQLGCGGSGGGGSGGGGSIQRTPKIQVYSRHPAENGKSNFLNCYVSGFHPSDIEVDLLKNGERIEKVEHSDLSFSKDWSFYLLYYTEFTPTEKDEYACRVNHVTLSQPKIVKWDRDMGGGGSGGGGSGGGGSGGGGSGSHSMRYFSAAVSRPGRGEPRFIAMGYVDDTQFVRFDSDAASPRMEPRAPWVEQEGPEYWDEETRNTKAHAQTDRVNLGTLRGCYNQSEAGSHTLQWMIGCDVGSDGRLLRGYEQYAYDGKDYLALNEDLRSWTAADTAAQISKRKCEAAHVAEQRRAYLEGTCVEWLRRYLENGKETLQRADPPKTHVTHHPVSDHEATLRCWALGFYPAEITLTWQRDGEDQTQDVELVETRPAGDGTFQKWAAVVVPSGEEQRYTCHVQHEGLPEPLTLRWKGGGLNDIFEAQKIEWHEHHHHHH

SEQ ID NO: 27 - protein, 441 aa, mus musculus
TYQRTRALVGCGGSGGGGSGGGGSIQKTPQIQVYSRHPPENGKPNILNCYVTQFHPPHIEIQMLKNGKKIPKVEMSDMSFSKDWSFYILAHTEFTPTETDTYACRVKHDSMAEPKTVYWDRDMGGGGSGGGGSGGGGSGGGGSGPHSLRYFVTAVSRPGLGEPRFIAVGYVDDTQFVRFDSDADNPRFEPRAPWMEQEGPEYWEEQTQRAKSDEQWFRVSLRTAQRCYNQSKGGSHTFQRMFGCDVGSDWRLLRGYQQFAYDGRDYIALNEDLKTWTAADTAALITRRKWEQAGDAEYYRAYLEGECVEWLRRYLELGNETLLRTDSPKAHVTYHPRSQVDVTLRCWALGFYPADITLTWQLNGEDLTQDMELVETRPAGDGTFQKWAAVVVPLGKEQNYTCHVHHKGLPEPLTLRWKGGGLNDIFEAQKIEWHEHHHHHH

SEQ ID NO: 28 - protein, 441 aa, Artificial
  exemplary human HLA-G/ mouse H2Kd ß2M MHC class I complex wherein the positions specific for human HLA-G are grafted onto the mouse H2Kd framework
TYQRTRALVGCGGSGGGGSGGGGSIQKTPQIQVYSRHPPENGKPNILNCYVTQFHPPHIEIQMLKNGKKIPKVEMSDMSFSKDWSFYILAHTEFTPTETDTYACRVKHDSMAEPKTVYWDRDMGGGGSGGGGSGGGGSGGGGSGPHSLRYFVTAVSRPGLGEPRFIAVGYVDDTQFVRFDSDSASPRFEPRAPWVEQEGPEYWEEQTQRAKSDEQWFRMSLQTARGCYNQSEASSHTFQRMFGCDLGSDGRLLRGYQQFAYDGRDYIALNEDLRSWTAADTAALITKRKWEAANDAEYYRAYLEGECVEWLHRYLENGKEMLQRTDSPKAHVTHHPVFDYEATLRCWALGFYPAEIILTWQLNGEDLTQDVELVETRPAGDGTFQKWAAVVVPSGKEQNYTCHVQHEGLPEPLMLRWKGGGLNDIFEAQKIEWHEHHHHHH

SEQ ID NO: 29 - protein, 440 aa, rat
AQFSASASRGCGGSGGGGSGGGGSIQKTPQIQVYSRHPPENGKPNFLNCYVSQFHPPQIEIELLKNGKKIPNIEMSDLSFSKDWSFYILAHTEFTPTETDVYACRVKHVTLKEPKTVTWDRDMGGGGSGGGGSGGGGSGGGGSGSHSLRYFYTAVSRPGLGEPRFIAVGYVDDTEFVRFDSDAENPRMEPRARWMEREGPEYWEQQTRIAKEWEQIYRVDLRTLRGCYNQSEGGSHTIQEMYGCDVGSDGSLLRGYRQDAYDGRDYIALNEDLKTWTAADFAAQITRNKWERARYAERLRAYLEGTCVEWLSRYLELGKETLLRSDPPEAHVTLHPRPEGDVTLRCWALGFYPADITLTWQLNGEDLTQDMELVETRPAGDGTFQKWASVVVPLGKEQNYTCRVEHEGLPKPLSQRWGSGLNDIFEAQKIEWHEHHHHHH

SEQ ID NO: 30 - protein, 440 aa, Artificial
  exemplary human HLA-G/ rat RT1A ß2M MHC class I complex wherein the positions specific for human HLA-G are grafted onto the rat RT1A framework
AQFSASASRGCGGSGGGGSGGGGSIQKTPQIQVYSRHPPENGKPNFLNCYVSQFHPPQIEIELLKNGKKIPNIEMSDLSFSKDWSFYILAHTEFTPTETDVYACRVKHVTLKEPKTVTWDRDMGGGGSGGGGSGGGGSGGGGSGSHSLRYFYTAVSRPGLGEPRFIAVGYVDDTEFVRFDSDSASPRMEPRAPWVEQEGPEYWEQQTRIAKEWEQIYRMDLQTLRGCYNQSEASSHTIQEMYGCDLGSDGRLLRGYRQDAYDGRDYIALNEDLRSWTAADFAAQITKRKWEAANYAERLRAYLEGTCVEWLHRYLENGKEMLQRADPPEAHVTHHPVFDYEATLRCWALGFYPAEIILTWQLNGEDLTQDVELVETRPAGDGTFQKWASVVVPSGKEQNYTCRVQHEGLPKPLMLRWGSGLNDIFEAQKIEWHEHHHHHH

SEQ ID NO: 31 - protein, 33 aa, Artificial
  linker and his-Tag
GGGGSGGGGSGSGLNDIFEAQKIEWHEHHHHHH

SEQ ID NO: 32 - protein, 9 aa, Artificial
  peptide
VLDFAPPGA

SEQ ID NO: 33 - protein, 107 aa, Homo Sapiens [sequence omitted]

SEQ ID NO: 34 - protein, 105 aa, Homo Sapiens
QPKAAPSVTLFPPSSEELQANKATLVCLISDFYPGAVTVAWKADSSPVKAGVETTTPSKQSNNKYAASSYLSLTPEQWKSHRSYSCQVTHEGSTVEKTVAPTECS

SEQ ID NO: 35 - protein, 328 aa, Homo Sapiens
ASTKGPSVFPLAPSSKSTSGGTAALGCLVKDYFPEPVTVSWNSGALTSGVHTFPAVLQSSGLYSLSSVVTVPSSSLGTQTYICNVNHKPSNTKVDKKVEPKSCDKTHTCPPCPAPELLGGPSVFLFPPKPKDTLMISRTPEVTCVVVDVSHEDPEVKFNWYVDGVEVHNAKTKPREEQYNSTYRVVSVLTVLHQDWLNGKEYKCKVSNKALPAPIEKTISKAKGQPREPQVYTLPPSRDELTKNQVSLTCLVKGFYPSDIAVEWESNGQPENNYKTTPPVLDSDGSFFLYSKLTVDKSRWQQGNVFSCSVMHEALHNHYTQKSLSLSP

SEQ ID NO: 36 - protein, 328 aa, homo sapiens
ASTKGPSVFPLAPSSKSTSGGTAALGCLVKDYFPEPVTVSWNSGALTSGVHTFPAVLQSSGLYSLSSVVTVPSSSLGTQTYICNVNHKPSNTKVDKKVEPKSCDKTHTCPPCPAPEAAGGPSVFLFPPKPKDTLMISRTPEVTCVVVDVSHEDPEVKFNWYVDGVEVHNAKTKPREEQYNSTYRVVSVLTVLHQDWLNGKEYKCKVSNKALGAPIEKTISKAKGQPREPQVYTLPPSRDELTKNQVSLTCLVKGFYPSDIAVEWESNGQPENNYKTTPPVLDSDGSFFLYSKLTVDKSRWQQGNVFSCSVMHEALHNHYTQKSLSLSP

SEQ ID NO: 37 - protein, 325 aa, Homo Sapiens
ASTKGPSVFPLAPCSRSTSESTAALGCLVKDYFPEPVTVSWNSGALTSGVHTFPAVLQSSGLYSLSSVVTVPSSSLGTKTYTCNVDHKPSNTKVDKRVESKYGPPCPSCPAPEFLGGPSVFLFPPKPKDTLMISRTPEVTCVVVDVSQEDPEVQFNWYVDGVEVHNAKTKPREEQFNSTYRVVSVLTVLHQDWLNGKEYKCKVSNKGLPSSIEKTISKAKGQPREPQVYTLPPSQEEMTKNQVSLTCLVKGFYPSDIAVEWESNGQPENNYKTTPPVLDSDGSFFLYSRLTVDKSRWQEGNVFSCSVMHEALHNHYTQKSLSLSL

SEQ ID NO: 38 - protein, 122 aa, rat
EVQLVETGGGLVQSGRSLKLSCVASGFTFNDYWMTWTRQAPGKGLEWVASITNSGGRTYYLDSVRGRFTISRDDAQNTLYLQMNSLRSEDTATYYCTKERIYLTAYWFFDFWGPGTMVTVSS

SEQ ID NO: 39 - protein, 106 aa, rat
DTILTQSPALAVSPGERVTISCRASESVSTLIHWYQQKPGQRPKLLIYLASHLESGVPARFSGSGSGTDFTLTIDPVEADDTATYYCQQSWNEPRTFGGGTKLELK